European Patent Application EP 4 581 940 A1, published July 9, 2025. Title: Novel Lactiplantibacillus plantarum SKO-001 and use thereof. Applicant: Kolmar BNH. The sequence listing filed with the application follows.

SEQUENCE LISTING (1 sequence)

SEQ ID NO: 1 - RNA, 1489 nt, Lactiplantibacillus plantarum
  source 1..1489: mol_type = genomic RNA
gacgaacgctggcggcgtgcctaatacatgcaagtcgaacgaactctggtattgattggtgcttgcatcatgatttacatttgagtgagtggcgaactggtgagtaacacgtgggaaacctgcccagaagcgggggataacacctggaaacagatgctaataccgcataacaacttggaccgcatggtccgagcttgaaagatggcttcggctatcacttttggatggtcccgcggcgtattagctagatggtggggtaacggctcaccatggcaatgatacgtagccgacctgagagggtaatcggccacattgggactgagacacggcccaaactcctacgggaggcagcagtagggaatcttccacaatggacgaaagtctgatggagcaacgccgcgtgagtgaagaagggtttcggctcgtaaaactctgttgttaaagaagaacatatctgagagtaactgttcaggtattgacggtatttaaccagaaagccacggctaactacgtgccagcagccgcggtaatacgtaggtggcaagcgttgtccggatttattgggcgtaaagcgagcgcaggcggttttttaagtctgatgtgaaagccttcggctcaaccgaagaagtgcatcggaaactgggaaacttgagtgcagaagaggacagtggaactccatgtgtagcggtgaaatgcgtagatatatggaagaacaccagtggcgaaggcggctgtctggtctgtaactgacgctgaggctcgaaagtatgggtagcaaacaggattagataccctggtagtccataccgtaaacgatgaatgctaagtgttggagggtttccacccttcagtgctgcagctaacgcattaagcattccgcctggggagtacggccgcaaggctgaaactcaaaggaattgacgggggcccgcacaagcggtggagcatgtggtttaattcgaagctacgcgaagaaccttaccaggtcttgacatactatgcaaatctaagagattagacgttcccttcggggacatggatacaggtggtgcatggttgtcgtcagctcgtgtcgtgagatgttgggttaagtcccgcaacgagcgcaacccttattatcagttgccagcattaagttgggcactctggtgagactgccggtgacaaaccggaggaaggtggggatgacgtcaaatcatcatgccccttatgacctgggctacacacgtgctacaatggatggtacaacgagttgcgaactcgcgagagtaagctaatctcttaaagccattctcagttcggattgtaggctgcaactcgcctacatgaagtcggaatcgctagtaatcgcggatcagcatgccgcggtgaatacgttcccgggccttgtacacaccgcccgtcacaccatgagagtttgtaacacccaaagtcggtggggtaaccttttaggaaccagccgcctaaggtgggacagatgattagggtg